European Patent Application EP 4 421 169 A1, published August 28, 2024. Title: Nucleic acid test method and Inspection kit. Applicant: FUJIFILM Corporation. The sequence listing filed with the application follows.

SEQUENCE LISTING (3 sequences)

SEQ ID NO: 1 - DNA, 29 bp, synthetic construct
  misc_feature 1..29: note = Forward primer
  source 1..29: mol_type = other DNA
ccmaggtcgaaacgtaygttctctctatc

SEQ ID NO: 2 - DNA, 32 bp, synthetic construct
  misc_feature 1..32: note = Reverse primer
  source 1..32: mol_type = other DNA
tgacagratyggtcttgtctttagccaytcca

SEQ ID NO: 3 - DNA, 22 bp, synthetic construct
  misc_feature 1..22: note = Probe
  modified_base 1: mod_base = OTHER; note = FAM is attached to a
  modified_base 22: mod_base = OTHER; note = MGB is attached to g
  source 1..22: mol_type = other DNA
atytcggctttgagggggcctg